European Patent Application EP 4 810 052 A2, published September 23, 2026. Title: hCRHR2 selective polypeptides. Applicant: Gubra A/S. The sequence listing filed with the application follows.

SEQUENCE LISTING (262 sequences)

SEQ ID NO: 1 - protein, 38 aa, Homo sapiens
IVLSLDVPIGLLQILLEQARARAAREQATTNARILARV

SEQ ID NO: 2 - protein, 38 aa, synthetic construct
  LIPID 29: note = C20DA-gGlu-gGlu-OEG-OEG
IVLSLDVPIGLLQILLEQARARAAREQAKTNARILARV

SEQ ID NO: 3 - protein, 38 aa, synthetic construct
  LIPID 29: note = C20DA-gGlu-gGlu-OEG-OEG
IVLSLDVPIGLLQILLEQARARAAREQAKTNAEILAEV

SEQ ID NO: 4 - protein, 38 aa, synthetic construct
  LIPID 30: note = C20DA-gGlu-gGlu-OEG-OEG
IVLSLDVPIGLLQILLEQARARAAREQATKNAEILAEV

SEQ ID NO: 5 - protein, 38 aa, synthetic construct
  SITE 1: note = MeIle
  LIPID 29: note = C20DA-gGlu-gGlu-OEG-OEG
XVLSLDVPIGLLQILLEQARARAAREQAKTNAEILAEV

SEQ ID NO: 6 - protein, 38 aa, synthetic construct
  SITE 1: note = MeIle
  LIPID 30: note = C20DA-gGlu-gGlu-OEG-OEG
XVLSLDVPIGLLQILLEQARARAAREQATKNAEILAEV

SEQ ID NO: 7 - protein, 38 aa, synthetic construct
  LIPID 29: note = C20DA-gGlu-gGlu-OEG-OEG
PVLSLDVPIGLLQILLEQARARAAREQAKTNAEILAEV

SEQ ID NO: 8 - protein, 38 aa, synthetic construct; identical to SEQ ID NO: 5
  SITE 1: note = N-acetyl-L-isoleucine
  LIPID 29: note = C20DA-gGlu-gGlu-OEG-OEG

SEQ ID NO: 9 - protein, 38 aa, synthetic construct
  SITE 1: note = MeIle
  LIPID 29: note = C20DA-gGlu-gGlu-OEG-OEG
XVLSLDVPIGLLQILLEQEKQEKEKQQAKTNAQILAQV

SEQ ID NO: 10 - protein, 38 aa, synthetic construct
  SITE 1: note = MeIle
  LIPID 29: note = C20DA-gGlu-gGlu-OEG-OEG
XVTSLDVPIGLLQILLEQEKQEKEKQQAKTNAEILAQV

SEQ ID NO: 11 - protein, 39 aa, synthetic construct
  LIPID 1: note = C20DA-gGlu-gGlu-gGlu-OEG-OEG
KIVLSLDVPIGLLQILLEQARARAAREQATTNAEILAEV

SEQ ID NO: 12 - protein, 38 aa, synthetic construct
  LIPID 29: note = C20DA-gGlu-gGlu-OEG-OEG
IVLSLDVPIGLLQILLEQARARAAREQAKTNLEILAEV

SEQ ID NO: 13 - protein, 38 aa, synthetic construct
  LIPID 29: note = C20DA-gGlu-gGlu-OEG-OEG
IVLSLDVPIGLLQILLEQARARAAREQAKTNIEILAEV

SEQ ID NO: 14 - protein, 38 aa, synthetic construct
  LIPID 29: note = C20DA-gGlu-gGlu-OEG-OEG
IVLSLDVPIGLLQILLEQARARAAREQAKTNVEILAEV

SEQ ID NO: 15 - protein, 38 aa, synthetic construct
  SITE 32: note = Aib
  LIPID 29: note = C20DA-gGlu-gGlu-OEG-OEG
IVLSLDVPIGLLQILLEQARARAAREQAKTNXEILAEV

SEQ ID NO: 16 - protein, 38 aa, synthetic construct
  SITE 1: note = MeIle
  SITE 32: note = Aib
  LIPID 29: note = C20DA-gGlu-gGlu-OEG-OEG
XVLSLDVPIGLLQILLEQARARAAREQAKTNXEILAEV

SEQ ID NO: 17 - protein, 38 aa, synthetic construct
  LIPID 29: note = C20DA-gGlu-gGlu-OEG-OEG
IVLSLDVPIGLLQILLEQARARAAREQAKENAEILAEV

SEQ ID NO: 18 - protein, 38 aa, synthetic construct
  SITE 1: note = MeIle
  LIPID 29: note = C20DA-gGlu-gGlu-OEG-OEG
XVLSLDVPIGLLQILLEQARARAAREQAKENAEILAEV

SEQ ID NO: 19 - protein, 38 aa, synthetic construct
  SITE 30: note = Aib
  LIPID 29: note = C20DA-gGlu-gGlu-OEG-OEG
IVLSLDVPIGLLQILLEQARARAAREQAKXNAEILAEV

SEQ ID NO: 20 - protein, 38 aa, synthetic construct
  SITE 1: note = MeIle
  SITE 30: note = Aib
  LIPID 29: note = C20DA-gGlu-gGlu-OEG-OEG
XVLSLDVPIGLLQILLEQARARAAREQAKXNAEILAEV

SEQ ID NO: 21 - protein, 38 aa, synthetic construct
  LIPID 29: note = C20DA-gGlu-gGlu-OEG-OEG
IVLSLDVPIGLLQILLEQARAESARERAKTNAEILAEI

SEQ ID NO: 22 - protein, 38 aa, synthetic construct
  SITE 35: note = Nle
  LIPID 29: note = C20DA-gGlu-gGlu-OEG-OEG
IVLSLDVPIGLLQILLEQARAESARERAKTNAEIXAEI

SEQ ID NO: 23 - protein, 38 aa, synthetic construct
  LIPID 29: note = C20DA-gGlu-gGlu-OEG-OEG
IVLSLDVPIGLLQILLEQARAEAAREQAKTNAEILAEI

SEQ ID NO: 24 - protein, 38 aa, synthetic construct
  SITE 35: note = Nle
  LIPID 29: note = C20DA-gGlu-gGlu-OEG-OEG
IVLSLDVPIGLLQILLEQARAEAAREQAKTNAEIXAEI

SEQ ID NO: 25 - protein, 38 aa, synthetic construct
  LIPID 29: note = C20DA-gGlu-gGlu-OEG-OEG
IVLSLDVPIGLLQILLEQARAEAAREQAKTNAEILAEV

SEQ ID NO: 26 - protein, 38 aa, synthetic construct
  SITE 35: note = Nle
  LIPID 29: note = C20DA-gGlu-gGlu-OEG-OEG
IVLSLDVPIGLLQILLEQARAEAAREQAKTNAEIXAEV

SEQ ID NO: 27 - protein, 38 aa, synthetic construct
  LIPID 29: note = C20DA-gGlu-gGlu-OEG-OEG
IVLSLDVPIGLLQILLEQARARAARQQAKTNAEILAEI

SEQ ID NO: 28 - protein, 38 aa, synthetic construct
  SITE 35: note = Nle
  LIPID 29: note = C20DA-gGlu-gGlu-OEG-OEG
IVLSLDVPIGLLQILLEQARARAARQQAKTNAEIXAEI

SEQ ID NO: 29 - protein, 38 aa, synthetic construct
  LIPID 29: note = C20DA-gGlu-gGlu-OEG-OEG
IVLSLDVPIGLLQILLEQARARQAREQAKTNAEILAEI

SEQ ID NO: 30 - protein, 38 aa, synthetic construct
  SITE 35: note = Nle
  LIPID 29: note = C20DA-gGlu-gGlu-OEG-OEG
IVLSLDVPIGLLQILLEQARARQAREQAKTNAEIXAEI

SEQ ID NO: 31 - protein, 38 aa, synthetic construct
  LIPID 29: note = C20DA-gGlu-gGlu-OEG-OEG
IVLSLDVPIGLLQILLEQARAQAQREQAKTNAEILAEV

SEQ ID NO: 32 - protein, 38 aa, synthetic construct
  SITE 35: note = Nle
  LIPID 29: note = C20DA-gGlu-gGlu-OEG-OEG
IVLSLDVPIGLLQILLEQARAQAQREQAKTNAEIXAEV

SEQ ID NO: 33 - protein, 38 aa, synthetic construct
  LIPID 29: note = C20DA-gGlu-gGlu-OEG-OEG
IVLSLDVPIGLLQILLEQARARAQREEAKTNAEILAEV

SEQ ID NO: 34 - protein, 38 aa, synthetic construct
  SITE 35: note = Nle
  LIPID 29: note = C20DA-gGlu-gGlu-OEG-OEG
IVLSLDVPIGLLQILLEQARARAQREEAKTNAEIXAEV

SEQ ID NO: 35 - protein, 38 aa, synthetic construct
  LIPID 29: note = C20DA-gGlu-gGlu-OEG-OEG
IVLSLDVPIGLLQILLEQARARSAREQAKTNAEILAEI

SEQ ID NO: 36 - protein, 38 aa, synthetic construct
  SITE 35: note = Nle
  LIPID 29: note = C20DA-gGlu-gGlu-OEG-OEG
IVLSLDVPIGLLQILLEQARARSAREQAKTNAEIXAEI

SEQ ID NO: 37 - protein, 38 aa, synthetic construct
  LIPID 29: note = C20DA-gGlu-gGlu-OEG-OEG
IVLSLDVPIGLLQILLEQARARALRQEAKTNAEILAEV

SEQ ID NO: 38 - protein, 38 aa, synthetic construct
  SITE 35: note = Nle
  LIPID 29: note = C20DA-gGlu-gGlu-OEG-OEG
IVLSLDVPIGLLQILLEQARARALRQEAKTNAEIXAEV

SEQ ID NO: 39 - protein, 38 aa, synthetic construct
  LIPID 29: note = C20DA-gGlu-gGlu-OEG-OEG
IVLSLDVPIGLLQILLEQARARALREQAKTNAEILAEV

SEQ ID NO: 40 - protein, 38 aa, synthetic construct
  SITE 35: note = Nle
  LIPID 29: note = C20DA-gGlu-gGlu-OEG-OEG
IVLSLDVPIGLLQILLEQARARALREQAKTNAEIXAEV

SEQ ID NO: 41 - protein, 38 aa, synthetic construct
  LIPID 29: note = C20DA-gGlu-gGlu-OEG-OEG
IVLSLDVPIGLLQILLEQARAESAREQAKTNAEILAEV

SEQ ID NO: 42 - protein, 38 aa, synthetic construct
  SITE 35: note = Nle
  LIPID 29: note = C20DA-gGlu-gGlu-OEG-OEG
IVLSLDVPIGLLQILLEQARAESAREQAKTNAEIXAEV

SEQ ID NO: 43 - protein, 38 aa, synthetic construct
  LIPID 29: note = C20DA-gGlu-gGlu-OEG-OEG
IVLSLDVPIGLLQILLEQARAQAAREQAKTNAEILAEI

SEQ ID NO: 44 - protein, 38 aa, synthetic construct
  SITE 35: note = Nle
  LIPID 29: note = C20DA-gGlu-gGlu-OEG-OEG
IVLSLDVPIGLLQILLEQARAQAAREQAKTNAEIXAEI

SEQ ID NO: 45 - protein, 38 aa, synthetic construct
  SITE 35: note = Nle
  LIPID 29: note = C20DA-gGlu-gGlu-OEG-OEG
IVLSLDVPIGLLQILLEQARARAAREQAKTNAEIXAEV

SEQ ID NO: 46 - protein, 38 aa, synthetic construct
  LIPID 29: note = C20DA-gGlu-gGlu-OEG-OEG
IVLSLDVPIGLLQILLEQARARAQRQQAKTNAEILAEV

SEQ ID NO: 47 - protein, 38 aa, synthetic construct
  SITE 35: note = Nle
  LIPID 29: note = C20DA-gGlu-gGlu-OEG-OEG
IVLSLDVPIGLLQILLEQARARAQRQQAKTNAEIXAEV

SEQ ID NO: 48 - protein, 38 aa, synthetic construct
  LIPID 29: note = C20DA-gGlu-gGlu-OEG-OEG
IVLSLDVPIGLLQILLEQARAQAARERAKTNAEILAEV

SEQ ID NO: 49 - protein, 38 aa, synthetic construct
  SITE 35: note = Nle
  LIPID 29: note = C20DA-gGlu-gGlu-OEG-OEG
IVLSLDVPIGLLQILLEQARAQAARERAKTNAEIXAEV

SEQ ID NO: 50 - protein, 38 aa, synthetic construct
  LIPID 29: note = C20DA-gGlu-gGlu-OEG-OEG
IVLSLDVPIGLLQILLEQARARALREEAKTNAEILAEV

SEQ ID NO: 51 - protein, 38 aa, synthetic construct
  SITE 35: note = Nle
  LIPID 29: note = C20DA-gGlu-gGlu-OEG-OEG
IVLSLDVPIGLLQILLEQARARALREEAKTNAEIXAEV

SEQ ID NO: 52 - protein, 38 aa, synthetic construct
  LIPID 29: note = C20DA-gGlu-gGlu-OEG-OEG
IVLSLDVPIGLLQILLEQARARQAREQAKTNAEILAEV

SEQ ID NO: 53 - protein, 38 aa, synthetic construct
  SITE 35: note = Nle
  LIPID 29: note = C20DA-gGlu-gGlu-OEG-OEG
IVLSLDVPIGLLQILLEQARARQAREQAKTNAEIXAEV

SEQ ID NO: 54 - protein, 38 aa, synthetic construct
  LIPID 29: note = C20DA-gGlu-gGlu-OEG-OEG
IVLSLDVPIGLLQILLEQARAQAARQQAKTNAEILAEV

SEQ ID NO: 55 - protein, 38 aa, synthetic construct
  SITE 35: note = Nle
  LIPID 29: note = C20DA-gGlu-gGlu-OEG-OEG
IVLSLDVPIGLLQILLEQARAQAARQQAKTNAEIXAEV

SEQ ID NO: 56 - protein, 38 aa, synthetic construct
  LIPID 29: note = C20DA-gGlu-gGlu-OEG-OEG
IVLSLDVPIGLLQILLEQARARAQREQAKTNAEILAEV

SEQ ID NO: 57 - protein, 38 aa, synthetic construct
  SITE 35: note = Nle
  LIPID 29: note = C20DA-gGlu-gGlu-OEG-OEG
IVLSLDVPIGLLQILLEQARARAQREQAKTNAEIXAEV

SEQ ID NO: 58 - protein, 38 aa, synthetic construct
  LIPID 29: note = C20DA-gGlu-gGlu-OEG-OEG
IVLSLDVPIGLLQILLEQARAEALRQQAKTNAEILAEV

SEQ ID NO: 59 - protein, 38 aa, synthetic construct
  SITE 35: note = Nle
  LIPID 29: note = C20DA-gGlu-gGlu-OEG-OEG
IVLSLDVPIGLLQILLEQARAEALRQQAKTNAEIXAEV

SEQ ID NO: 60 - protein, 38 aa, synthetic construct
  LIPID 29: note = C20DA-gGlu-gGlu-OEG-OEG
IVLSLDVPIGLLQILLEQARARSAREQAKTNAEILAEV

SEQ ID NO: 61 - protein, 38 aa, synthetic construct
  SITE 35: note = Nle
  LIPID 29: note = C20DA-gGlu-gGlu-OEG-OEG
IVLSLDVPIGLLQILLEQARARSAREQAKTNAEIXAEV

SEQ ID NO: 62 - protein, 38 aa, synthetic construct
  LIPID 29: note = C20DA-gGlu-gGlu-OEG-OEG
IVLSLDVPIGLLQILLEQARAQAAREQAKTNAEILAEV

SEQ ID NO: 63 - protein, 38 aa, synthetic construct
  SITE 35: note = Nle
  LIPID 29: note = C20DA-gGlu-gGlu-OEG-OEG
IVLSLDVPIGLLQILLEQARAQAAREQAKTNAEIXAEV

SEQ ID NO: 64 - protein, 38 aa, synthetic construct
  LIPID 29: note = C20DA-gGlu-gGlu-OEG-OEG
IVLSLDVPIGLLQILLEQARARAQREQAKTNAEILAEI

SEQ ID NO: 65 - protein, 38 aa, synthetic construct
  SITE 35: note = Nle
  LIPID 29: note = C20DA-gGlu-gGlu-OEG-OEG
IVLSLDVPIGLLQILLEQARARAQREQAKTNAEIXAEI

SEQ ID NO: 66 - protein, 38 aa, synthetic construct
  LIPID 29: note = C20DA-gGlu-gGlu-OEG-OEG
IVLSLDVPIGLLQILLEQARARAARERAKTNAEILAEV

SEQ ID NO: 67 - protein, 38 aa, synthetic construct
  SITE 35: note = Nle
  LIPID 29: note = C20DA-gGlu-gGlu-OEG-OEG
IVLSLDVPIGLLQILLEQARARAARERAKTNAEIXAEV

SEQ ID NO: 68 - protein, 38 aa, synthetic construct
  LIPID 29: note = C20DA-gGlu-gGlu-OEG-OEG
IVLSLDVPIGLLQILLEQARARAAREQAKTNAEILAEI

SEQ ID NO: 69 - protein, 38 aa, synthetic construct
  SITE 35: note = Nle
  LIPID 29: note = C20DA-gGlu-gGlu-OEG-OEG
IVLSLDVPIGLLQILLEQARARAAREQAKTNAEIXAEI

SEQ ID NO: 70 - protein, 38 aa, synthetic construct
  LIPID 29: note = C20DA-gGlu-gGlu-OEG-OEG
IVLSLDVPIGLLQILLEQARARSQREEAKTNAEILAEV

SEQ ID NO: 71 - protein, 38 aa, synthetic construct
  SITE 35: note = Nle
  LIPID 29: note = C20DA-gGlu-gGlu-OEG-OEG
IVLSLDVPIGLLQILLEQARARSQREEAKTNAEIXAEV

SEQ ID NO: 72 - protein, 38 aa, synthetic construct
  LIPID 29: note = C20DA-gGlu-gGlu-OEG-OEG
IVLSLDVPIGLLQILLEQARARQLREQAKTNAEILAEV

SEQ ID NO: 73 - protein, 38 aa, synthetic construct
  SITE 35: note = Nle
  LIPID 29: note = C20DA-gGlu-gGlu-OEG-OEG
IVLSLDVPIGLLQILLEQARARQLREQAKTNAEIXAEV

SEQ ID NO: 74 - protein, 38 aa, synthetic construct
  LIPID 29: note = C20DA-gGlu-gGlu-OEG-OEG
IVLSLDVPIGLLQILLEQARARAAREEAKTNAEILAEI

SEQ ID NO: 75 - protein, 38 aa, synthetic construct
  SITE 35: note = Nle
  LIPID 29: note = C20DA-gGlu-gGlu-OEG-OEG
IVLSLDVPIGLLQILLEQARARAAREEAKTNAEIXAEI

SEQ ID NO: 76 - protein, 38 aa, synthetic construct
  SITE 8: note = (2S,4S)-L-Pro(4-NH2)-OH
  LIPID 29: note = C20DA-gGlu-gGlu-OEG-OEG
IVLSLDVXIGLLQILLEQARARVAREQAKTNAEILAEV

SEQ ID NO: 77 - protein, 38 aa, synthetic construct
  SITE 8: note = (2S,4S)-L-Pro(4-NH2)-OH
  SITE 35: note = Nle
  LIPID 29: note = C20DA-gGlu-gGlu-OEG-OEG
IVLSLDVXIGLLQILLEQARARVAREQAKTNAEIXAEV

SEQ ID NO: 78 - protein, 38 aa, synthetic construct
  SITE 7: note = L-cycloleucine
  LIPID 29: note = C20DA-gGlu-gGlu-OEG-OEG
IVLSLDXPIGLLQILLEQARARQAREQAKTNAEILAEV

SEQ ID NO: 79 - protein, 38 aa, synthetic construct
  SITE 7: note = L-cycloleucine
  SITE 35: note = Nle
  LIPID 29: note = C20DA-gGlu-gGlu-OEG-OEG
IVLSLDXPIGLLQILLEQARARQAREQAKTNAEIXAEV

SEQ ID NO: 80 - protein, 38 aa, synthetic construct
  SITE 8: note = (2S,4S)-L-Pro(4-F)-OH
  LIPID 29: note = C20DA-gGlu-gGlu-OEG-OEG
IVLSLDVXIGLLQILLTQARARAAREQAKTNAEILAEV

SEQ ID NO: 81 - protein, 38 aa, synthetic construct
  SITE 8: note = (2S,4S)-L-Pro(4-F)-OH
  SITE 35: note = Nle
  LIPID 29: note = C20DA-gGlu-gGlu-OEG-OEG
IVLSLDVXIGLLQILLTQARARAAREQAKTNAEIXAEV

SEQ ID NO: 82 - protein, 38 aa, synthetic construct
  LIPID 29: note = C20DA-gGlu-gGlu-OEG-OEG
IVLSLDVPIGLLQILLSQARARAAREQAKTNAEILAEV

SEQ ID NO: 83 - protein, 38 aa, synthetic construct
  SITE 35: note = Nle
  LIPID 29: note = C20DA-gGlu-gGlu-OEG-OEG
IVLSLDVPIGLLQILLSQARARAAREQAKTNAEIXAEV

SEQ ID NO: 84 - protein, 38 aa, synthetic construct; identical to SEQ ID NO: 76
  SITE 8: note = 4Hyp
  LIPID 29: note = C20DA-gGlu-gGlu-OEG-OEG

SEQ ID NO: 85 - protein, 38 aa, synthetic construct; identical to SEQ ID NO: 77
  SITE 8: note = 4Hyp
  SITE 35: note = Nle
  LIPID 29: note = C20DA-gGlu-gGlu-OEG-OEG

SEQ ID NO: 86 - protein, 38 aa, synthetic construct
  SITE 7: note = L-cycloleucine
  SITE 8: note = (2S,4S)-L-Pro(4-F)-OH
  LIPID 29: note = C20DA-gGlu-gGlu-OEG-OEG
IVLSLDXXIGLLQILLEQARARAAREQAKTNAEILAEV

SEQ ID NO: 87 - protein, 38 aa, synthetic construct
  SITE 7: note = L-cycloleucine
  SITE 8: note = (2S,4S)-L-Pro(4-F)-OH
  SITE 35: note = Nle
  LIPID 29: note = C20DA-gGlu-gGlu-OEG-OEG
IVLSLDXXIGLLQILLEQARARAAREQAKTNAEIXAEV

SEQ ID NO: 88 - protein, 38 aa, synthetic construct
  LIPID 29: note = C20DA-gGlu-gGlu-OEG-OEG
IVLSLDVPIGLLQILLSQARARAAREQAKTNAEILAEI

SEQ ID NO: 89 - protein, 38 aa, synthetic construct
  SITE 35: note = Nle
  LIPID 29: note = C20DA-gGlu-gGlu-OEG-OEG
IVLSLDVPIGLLQILLSQARARAAREQAKTNAEIXAEI

SEQ ID NO: 90 - protein, 38 aa, synthetic construct
  LIPID 29: note = C20DA-gGlu-gGlu-OEG-OEG
IVLSLDVPIGLLQILLEQARARVAREQAKTNAEILAEV

SEQ ID NO: 91 - protein, 38 aa, synthetic construct
  SITE 35: note = Nle
  LIPID 29: note = C20DA-gGlu-gGlu-OEG-OEG
IVLSLDVPIGLLQILLEQARARVAREQAKTNAEIXAEV

SEQ ID NO: 92 - protein, 38 aa, synthetic construct
  LIPID 29: note = C20DA-gGlu-gGlu-OEG-OEG
IVLSLDVPIGLLQILLTQARARQAREQAKTNAEILAEV

SEQ ID NO: 93 - protein, 38 aa, synthetic construct
  SITE 35: note = Nle
  LIPID 29: note = C20DA-gGlu-gGlu-OEG-OEG
IVLSLDVPIGLLQILLTQARARQAREQAKTNAEIXAEV

SEQ ID NO: 94 - protein, 38 aa, synthetic construct
  LIPID 29: note = C20DA-gGlu-gGlu-OEG-OEG
IVLSLDVPIGLLQILLSQARARIAREQAKTNAEILAEV

SEQ ID NO: 95 - protein, 38 aa, synthetic construct
  SITE 35: note = Nle
  LIPID 29: note = C20DA-gGlu-gGlu-OEG-OEG
IVLSLDVPIGLLQILLSQARARIAREQAKTNAEIXAEV

SEQ ID NO: 96 - protein, 38 aa, synthetic construct
  SITE 8: note = (2S,4S)-L-Pro(4-F)-OH
  LIPID 29: note = C20DA-gGlu-gGlu-OEG-OEG
IVLSLDVXIGLLQILLEQARARNAREQAKTNAEILAEV

SEQ ID NO: 97 - protein, 38 aa, synthetic construct
  SITE 8: note = (2S,4S)-L-Pro(4-F)-OH
  SITE 35: note = Nle
  LIPID 29: note = C20DA-gGlu-gGlu-OEG-OEG
IVLSLDVXIGLLQILLEQARARNAREQAKTNAEIXAEV

SEQ ID NO: 98 - protein, 38 aa, synthetic construct
  LIPID 29: note = C20DA-gGlu-gGlu-OEG-OEG
IVLSLDVPLGLLQILLEQARARAAREQAKTNAEILAEV

SEQ ID NO: 99 - protein, 38 aa, synthetic construct
  SITE 35: note = Nle
  LIPID 29: note = C20DA-gGlu-gGlu-OEG-OEG
IVLSLDVPLGLLQILLEQARARAAREQAKTNAEIXAEV

SEQ ID NO: 100 - protein, 38 aa, synthetic construct
  SITE 32: note = Aib
  SITE 35: note = Nle
  LIPID 29: note = C20DA-gGlu-gGlu-OEG-OEG
IVLSLDVPIGLLQILLEQARARAAREQAKTNXEIXAEI

SEQ ID NO: 101 - protein, 38 aa, synthetic construct
  SITE 1: note = MeIle
  SITE 35: note = Nle
  LIPID 29: note = C20DA-gGlu-gGlu-OEG-OEG
XVLSLDVPIGLLQILLSQARARAAREQAKENAEIXAEV

SEQ ID NO: 102 - protein, 38 aa, synthetic construct
  SITE 8: note = (2S,4S)-L-Pro(4-F)-OH
  LIPID 29: note = C20DA-gGlu-gGlu-OEG-OEG
IVLSLDVXIGLLQILLEQARARAAREQAKTNAEILAEV

SEQ ID NO: 103 - protein, 38 aa, synthetic construct
  SITE 8: note = (2S,4S)-L-Pro(4-F)-OH
  SITE 35: note = Nle
  LIPID 29: note = C20DA-gGlu-gGlu-OEG-OEG
IVLSLDVXIGLLQILLEQARARAAREQAKTNAEIXAEV

SEQ ID NO: 104 - protein, 38 aa, synthetic construct
  SITE 8: note = (2S,4S)-L-Pro(4-NH2)-OH
  LIPID 29: note = C20DA-gGlu-gGlu-OEG-OEG
IVLSLDVXIGLLQILLEQARARIAREQAKTNAEILAEV

SEQ ID NO: 105 - protein, 38 aa, synthetic construct
  SITE 8: note = (2S,4S)-L-Pro(4-NH2)-OH
  SITE 35: note = Nle
  LIPID 29: note = C20DA-gGlu-gGlu-OEG-OEG
IVLSLDVXIGLLQILLEQARARIAREQAKTNAEIXAEV

SEQ ID NO: 106 - protein, 38 aa, synthetic construct; identical to SEQ ID NO: 76
  SITE 8: note = (2S,4S)-L-Pro(4-F)-OH
  LIPID 29: note = C20DA-gGlu-gGlu-OEG-OEG

SEQ ID NO: 107 - protein, 38 aa, synthetic construct; identical to SEQ ID NO: 77
  SITE 8: note = (2S,4S)-L-Pro(4-F)-OH
  SITE 35: note = Nle
  LIPID 29: note = C20DA-gGlu-gGlu-OEG-OEG

SEQ ID NO: 108 - protein, 38 aa, synthetic construct
  SITE 7: note = L-cycloleucine
  LIPID 29: note = C20DA-gGlu-gGlu-OEG-OEG
IVLSLDXPIGLLQILLEQARARVAREQAKTNAEILAEV

SEQ ID NO: 109 - protein, 38 aa, synthetic construct
  SITE 7: note = L-cycloleucine
  SITE 35: note = Nle
  LIPID 29: note = C20DA-gGlu-gGlu-OEG-OEG
IVLSLDXPIGLLQILLEQARARVAREQAKTNAEIXAEV

SEQ ID NO: 110 - protein, 38 aa, synthetic construct
  SITE 7: note = L-cycloleucine
  LIPID 29: note = C20DA-gGlu-gGlu-OEG-OEG
IVLSLDXPIGLLQILLEQARARAAREQAKTNAEILAEV

SEQ ID NO: 111 - protein, 38 aa, synthetic construct
  SITE 7: note = L-cycloleucine
  SITE 35: note = Nle
  LIPID 29: note = C20DA-gGlu-gGlu-OEG-OEG
IVLSLDXPIGLLQILLEQARARAAREQAKTNAEIXAEV

SEQ ID NO: 112 - protein, 38 aa, synthetic construct
  LIPID 29: note = C20DA-gGlu-gGlu-OEG-OEG
IVLSLDVPIGLLQILLTQARARNAREQAKTNAEILAEV

SEQ ID NO: 113 - protein, 38 aa, synthetic construct
  SITE 35: note = Nle
  LIPID 29: note = C20DA-gGlu-gGlu-OEG-OEG
IVLSLDVPIGLLQILLTQARARNAREQAKTNAEIXAEV

SEQ ID NO: 114 - protein, 38 aa, synthetic construct
  LIPID 29: note = C20DA-gGlu-gGlu-OEG-OEG
IVLSLDVPIGLLQILLEQARARNAREQAKTNAEILAEV

SEQ ID NO: 115 - protein, 38 aa, synthetic construct
  SITE 35: note = Nle
  LIPID 29: note = C20DA-gGlu-gGlu-OEG-OEG
IVLSLDVPIGLLQILLEQARARNAREQAKTNAEIXAEV

SEQ ID NO: 116 - protein, 38 aa, synthetic construct
  SITE 8: note = (2S,4S)-L-Pro(4-NH2)-OH
  LIPID 29: note = C20DA-gGlu-gGlu-OEG-OEG
IVLSLDVXIGLLQILLEQARARQAREQAKTNAEILAEV

SEQ ID NO: 117 - protein, 38 aa, synthetic construct
  SITE 8: note = (2S,4S)-L-Pro(4-NH2)-OH
  SITE 35: note = Nle
  LIPID 29: note = C20DA-gGlu-gGlu-OEG-OEG
IVLSLDVXIGLLQILLEQARARQAREQAKTNAEIXAEV

SEQ ID NO: 118 - protein, 38 aa, synthetic construct
  SITE 1: note = MeIle
  SITE 30: note = Aib
  LIPID 29: note = C20DA-gGlu-gGlu-OEG-OEG
XVLSLDVPIGLLQILLAQARARAAREQAKXNAEILAEV

SEQ ID NO: 119 - protein, 38 aa, synthetic construct
  SITE 1: note = MeIle
  SITE 30: note = Aib
  SITE 35: note = Nle
  LIPID 29: note = C20DA-gGlu-gGlu-OEG-OEG
XVLSLDVPIGLLQILLAQARARAAREQAKXNAEIXAEV

SEQ ID NO: 120 - protein, 38 aa, synthetic construct
  SITE 1: note = MeIle
  SITE 30: note = Aib
  LIPID 29: note = C20DA-gGlu-gGlu-OEG-OEG
XVLSLDVPIGLLQILLDQARARAAREQAKXNAEILAEV

SEQ ID NO: 121 - protein, 38 aa, synthetic construct
  SITE 1: note = MeIle
  SITE 30: note = Aib
  SITE 35: note = Nle
  LIPID 29: note = C20DA-gGlu-gGlu-OEG-OEG
XVLSLDVPIGLLQILLDQARARAAREQAKXNAEIXAEV

SEQ ID NO: 122 - protein, 38 aa, synthetic construct
  SITE 1: note = MeIle
  SITE 30: note = Aib
  LIPID 29: note = C20DA-gGlu-gGlu-OEG-OEG
XVLSLDVPIGLLQILLGQARARAAREQAKXNAEILAEV

SEQ ID NO: 123 - protein, 38 aa, synthetic construct
  SITE 1: note = MeIle
  SITE 30: note = Aib
  SITE 35: note = Nle
  LIPID 29: note = C20DA-gGlu-gGlu-OEG-OEG
XVLSLDVPIGLLQILLGQARARAAREQAKXNAEIXAEV

SEQ ID NO: 124 - protein, 38 aa, synthetic construct
  SITE 1: note = MeIle
  SITE 30: note = Aib
  SITE 35: note = Nle
  LIPID 29: note = C20DA-gGlu-gGlu-OEG-OEG
XVLSLDVPIGLLQILLEQARARAAREQAKXNAEIXAEV

SEQ ID NO: 125 - protein, 38 aa, synthetic construct
  SITE 1: note = MeIle
  SITE 30: note = Aib
  LIPID 29: note = C20DA-gGlu-gGlu-OEG-OEG
XVLSLDVPIGLLQILLHQARARAAREQAKXNAEILAEV

SEQ ID NO: 126 - protein, 38 aa, synthetic construct
  SITE 1: note = MeIle
  SITE 30: note = Aib
  SITE 35: note = Nle
  LIPID 29: note = C20DA-gGlu-gGlu-OEG-OEG
XVLSLDVPIGLLQILLHQARARAAREQAKXNAEIXAEV

SEQ ID NO: 127 - protein, 38 aa, synthetic construct
  SITE 1: note = MeIle
  SITE 30: note = Aib
  LIPID 29: note = C20DA-gGlu-gGlu-OEG-OEG
XVLSLDVPIGLLQILLFQARARAAREQAKXNAEILAEV

SEQ ID NO: 128 - protein, 38 aa, synthetic construct
  SITE 1: note = MeIle
  SITE 30: note = Aib
  SITE 35: note = Nle
  LIPID 29: note = C20DA-gGlu-gGlu-OEG-OEG
XVLSLDVPIGLLQILLFQARARAAREQAKXNAEIXAEV

SEQ ID NO: 129 - protein, 38 aa, synthetic construct
  SITE 1: note = MeIle
  SITE 30: note = Aib
  LIPID 29: note = C20DA-gGlu-gGlu-OEG-OEG
XVLSLDVPIGLLQILLPQARARAAREQAKXNAEILAEV

SEQ ID NO: 130 - protein, 38 aa, synthetic construct
  SITE 1: note = MeIle
  SITE 30: note = Aib
  SITE 35: note = Nle
  LIPID 29: note = C20DA-gGlu-gGlu-OEG-OEG
XVLSLDVPIGLLQILLPQARARAAREQAKXNAEIXAEV

SEQ ID NO: 131 - protein, 38 aa, synthetic construct
  SITE 1: note = MeIle
  SITE 30: note = Aib
  LIPID 29: note = C20DA-gGlu-gGlu-OEG-OEG
XVLSLDVPIGLLQILLSQARARAAREQAKXNAEILAEV

SEQ ID NO: 132 - protein, 38 aa, synthetic construct
  SITE 1: note = MeIle
  SITE 30: note = Aib
  SITE 35: note = Nle
  LIPID 29: note = C20DA-gGlu-gGlu-OEG-OEG
XVLSLDVPIGLLQILLSQARARAAREQAKXNAEIXAEV

SEQ ID NO: 133 - protein, 38 aa, synthetic construct
  SITE 1: note = MeIle
  SITE 30: note = Aib
  LIPID 29: note = C20DA-gGlu-gGlu-OEG-OEG
XVLSLDVPIGLLQILLTQARARAAREQAKXNAEILAEV

SEQ ID NO: 134 - protein, 38 aa, synthetic construct
  SITE 1: note = MeIle
  SITE 30: note = Aib
  SITE 35: note = Nle
  LIPID 29: note = C20DA-gGlu-gGlu-OEG-OEG
XVLSLDVPIGLLQILLTQARARAAREQAKXNAEIXAEV

SEQ ID NO: 135 - protein, 38 aa, synthetic construct
  SITE 1: note = MeIle
  SITE 30: note = Aib
  LIPID 29: note = C20DA-gGlu-gGlu-OEG-OEG
XVLSLDVPIGLLQILLWQARARAAREQAKXNAEILAEV

SEQ ID NO: 136 - protein, 38 aa, synthetic construct
  SITE 1: note = MeIle
  SITE 30: note = Aib
  SITE 35: note = Nle
  LIPID 29: note = C20DA-gGlu-gGlu-OEG-OEG
XVLSLDVPIGLLQILLWQARARAAREQAKXNAEIXAEV

SEQ ID NO: 137 - protein, 38 aa, synthetic construct
  SITE 1: note = MeIle
  SITE 30: note = Aib
  LIPID 29: note = C20DA-gGlu-gGlu-OEG-OEG
XVLSLDVPIGLLQILLVQARARAAREQAKXNAEILAEV

SEQ ID NO: 138 - protein, 38 aa, synthetic construct
  SITE 1: note = MeIle
  SITE 30: note = Aib
  SITE 35: note = Nle
  LIPID 29: note = C20DA-gGlu-gGlu-OEG-OEG
XVLSLDVPIGLLQILLVQARARAAREQAKXNAEIXAEV

SEQ ID NO: 139 - protein, 38 aa, synthetic construct
  SITE 1: note = MeIle
  SITE 30: note = Aib
  LIPID 29: note = C20DA-gGlu-gGlu-OEG-OEG
XVLSLDVPIGLLQILLEQARARAAREQAKXNAEILAEI

SEQ ID NO: 140 - protein, 38 aa, synthetic construct
  SITE 1: note = MeIle
  SITE 30: note = Aib
  SITE 35: note = Nle
  LIPID 29: note = C20DA-gGlu-gGlu-OEG-OEG
XVLSLDVPIGLLQILLEQARARAAREQAKXNAEIXAEI

SEQ ID NO: 141 - protein, 38 aa, synthetic construct
  SITE 1: note = MeIle
  SITE 30: note = Aib
  LIPID 29: note = C20DA-gGlu-gGlu-OEG-OEG
XVLSLDVPIGLLQILLEQARARAAREQAKXNAEILAEL

SEQ ID NO: 142 - protein, 38 aa, synthetic construct
  SITE 1: note = MeIle
  SITE 30: note = Aib
  SITE 35: note = Nle
  LIPID 29: note = C20DA-gGlu-gGlu-OEG-OEG
XVLSLDVPIGLLQILLEQARARAAREQAKXNAEIXAEL

SEQ ID NO: 143 - protein, 38 aa, synthetic construct
  SITE 1: note = MeIle
  SITE 30: note = Aib
  SITE 38: note = Aib
  LIPID 29: note = C20DA-gGlu-gGlu-OEG-OEG
XVLSLDVPIGLLQILLEQARARAAREQAKXNAEILAEX

SEQ ID NO: 144 - protein, 38 aa, synthetic construct
  SITE 1: note = MeIle
  SITE 30: note = Aib
  SITE 35: note = Nle
  SITE 38: note = Aib
  LIPID 29: note = C20DA-gGlu-gGlu-OEG-OEG
XVLSLDVPIGLLQILLEQARARAAREQAKXNAEIXAEX

SEQ ID NO: 145 - protein, 38 aa, synthetic construct
  SITE 1: note = MeIle
  LIPID 29: note = C20DA-gGlu-gGlu-OEG-OEG
XVLSLDVPIGLLQILLSQARARAAREQAKANAEILAEV

SEQ ID NO: 146 - protein, 38 aa, synthetic construct
  SITE 1: note = MeIle
  SITE 35: note = Nle
  LIPID 29: note = C20DA-gGlu-gGlu-OEG-OEG
XVLSLDVPIGLLQILLSQARARAAREQAKANAEIXAEV

SEQ ID NO: 147 - protein, 38 aa, synthetic construct
  SITE 1: note = MeIle
  LIPID 29: note = C20DA-gGlu-gGlu-OEG-OEG
XVLSLDVPIGLLQILLSQARARAAREQAKQNAEILAEV

SEQ ID NO: 148 - protein, 38 aa, synthetic construct
  SITE 1: note = MeIle
  SITE 35: note = Nle
  LIPID 29: note = C20DA-gGlu-gGlu-OEG-OEG
XVLSLDVPIGLLQILLSQARARAAREQAKQNAEIXAEV

SEQ ID NO: 149 - protein, 38 aa, synthetic construct
  SITE 1: note = MeIle
  LIPID 29: note = C20DA-gGlu-gGlu-OEG-OEG
XVLSLDVPIGLLQILLSQARARAAREQAKGNAEILAEV

SEQ ID NO: 150 - protein, 38 aa, synthetic construct
  SITE 1: note = MeIle
  SITE 35: note = Nle
  LIPID 29: note = C20DA-gGlu-gGlu-OEG-OEG
XVLSLDVPIGLLQILLSQARARAAREQAKGNAEIXAEV

SEQ ID NO: 151 - protein, 38 aa, synthetic construct
  SITE 1: note = MeIle
  LIPID 29: note = C20DA-gGlu-gGlu-OEG-OEG
XVLSLDVPIGLLQILLSQARARAAREQAKHNAEILAEV

SEQ ID NO: 152 - protein, 38 aa, synthetic construct
  SITE 1: note = MeIle
  SITE 35: note = Nle
  LIPID 29: note = C20DA-gGlu-gGlu-OEG-OEG
XVLSLDVPIGLLQILLSQARARAAREQAKHNAEIXAEV

SEQ ID NO: 153 - protein, 38 aa, synthetic construct
  SITE 1: note = MeIle
  LIPID 29: note = C20DA-gGlu-gGlu-OEG-OEG
XVLSLDVPIGLLQILLSQARARAAREQAKINAEILAEV

SEQ ID NO: 154 - protein, 38 aa, synthetic construct
  SITE 1: note = MeIle
  SITE 35: note = Nle
  LIPID 29: note = C20DA-gGlu-gGlu-OEG-OEG
XVLSLDVPIGLLQILLSQARARAAREQAKINAEIXAEV

SEQ ID NO: 155 - protein, 38 aa, synthetic construct
  SITE 1: note = MeIle
  LIPID 29: note = C20DA-gGlu-gGlu-OEG-OEG
XVLSLDVPIGLLQILLSQARARAAREQAKLNAEILAEV

SEQ ID NO: 156 - protein, 38 aa, synthetic construct
  SITE 1: note = MeIle
  SITE 35: note = Nle
  LIPID 29: note = C20DA-gGlu-gGlu-OEG-OEG
XVLSLDVPIGLLQILLSQARARAAREQAKLNAEIXAEV

SEQ ID NO: 157 - protein, 38 aa, synthetic construct
  SITE 1: note = MeIle
  LIPID 29: note = C20DA-gGlu-gGlu-OEG-OEG
XVLSLDVPIGLLQILLSQARARAAREQAKFNAEILAEV

SEQ ID NO: 158 - protein, 38 aa, synthetic construct
  SITE 1: note = MeIle
  SITE 35: note = Nle
  LIPID 29: note = C20DA-gGlu-gGlu-OEG-OEG
XVLSLDVPIGLLQILLSQARARAAREQAKFNAEIXAEV

SEQ ID NO: 159 - protein, 38 aa, synthetic construct
  SITE 1: note = MeIle
  LIPID 29: note = C20DA-gGlu-gGlu-OEG-OEG
XVLSLDVPIGLLQILLSQARARAAREQAKPNAEILAEV

SEQ ID NO: 160 - protein, 38 aa, synthetic construct
  SITE 1: note = MeIle
  SITE 35: note = Nle
  LIPID 29: note = C20DA-gGlu-gGlu-OEG-OEG
XVLSLDVPIGLLQILLSQARARAAREQAKPNAEIXAEV

SEQ ID NO: 161 - protein, 38 aa, synthetic construct
  SITE 1: note = MeIle
  LIPID 29: note = C20DA-gGlu-gGlu-OEG-OEG
XVLSLDVPIGLLQILLSQARARAAREQAKSNAEILAEV

SEQ ID NO: 162 - protein, 38 aa, synthetic construct
  SITE 1: note = MeIle
  SITE 35: note = Nle
  LIPID 29: note = C20DA-gGlu-gGlu-OEG-OEG
XVLSLDVPIGLLQILLSQARARAAREQAKSNAEIXAEV

SEQ ID NO: 163 - protein, 38 aa, synthetic construct
  SITE 1: note = MeIle
  LIPID 29: note = C20DA-gGlu-gGlu-OEG-OEG
XVLSLDVPIGLLQILLSQARARAAREQAKTNAEILAEV

SEQ ID NO: 164 - protein, 38 aa, synthetic construct
  SITE 1: note = MeIle
  SITE 35: note = Nle
  LIPID 29: note = C20DA-gGlu-gGlu-OEG-OEG
XVLSLDVPIGLLQILLSQARARAAREQAKTNAEIXAEV

SEQ ID NO: 165 - protein, 38 aa, synthetic construct
  SITE 1: note = MeIle
  LIPID 29: note = C20DA-gGlu-gGlu-OEG-OEG
XVLSLDVPIGLLQILLSQARARAAREQAKWNAEILAEV

SEQ ID NO: 166 - protein, 38 aa, synthetic construct
  SITE 1: note = MeIle
  SITE 35: note = Nle
  LIPID 29: note = C20DA-gGlu-gGlu-OEG-OEG
XVLSLDVPIGLLQILLSQARARAAREQAKWNAEIXAEV

SEQ ID NO: 167 - protein, 38 aa, synthetic construct
  SITE 1: note = MeIle
  LIPID 29: note = C20DA-gGlu-gGlu-OEG-OEG
XVLSLDVPIGLLQILLSQARARAAREQAKYNAEILAEV

SEQ ID NO: 168 - protein, 38 aa, synthetic construct
  SITE 1: note = MeIle
  SITE 35: note = Nle
  LIPID 29: note = C20DA-gGlu-gGlu-OEG-OEG
XVLSLDVPIGLLQILLSQARARAAREQAKYNAEIXAEV

SEQ ID NO: 169 - protein, 38 aa, synthetic construct
  SITE 1: note = MeIle
  LIPID 29: note = C20DA-gGlu-gGlu-OEG-OEG
XVLSLDVPIGLLQILLSQARARAAREQAKVNAEILAEV

SEQ ID NO: 170 - protein, 38 aa, synthetic construct
  SITE 1: note = MeIle
  SITE 35: note = Nle
  LIPID 29: note = C20DA-gGlu-gGlu-OEG-OEG
XVLSLDVPIGLLQILLSQARARAAREQAKVNAEIXAEV

SEQ ID NO: 171 - protein, 38 aa, synthetic construct
  SITE 1: note = MeIle
  LIPID 29: note = C20DA-gGlu-gGlu-OEG-OEG
XVLSLDVPIGLLQILLSQARARAAREQAKTNREILAEV

SEQ ID NO: 172 - protein, 38 aa, synthetic construct
  SITE 1: note = MeIle
  SITE 35: note = Nle
  LIPID 29: note = C20DA-gGlu-gGlu-OEG-OEG
XVLSLDVPIGLLQILLSQARARAAREQAKTNREIXAEV

SEQ ID NO: 173 - protein, 38 aa, synthetic construct
  SITE 1: note = MeIle
  LIPID 29: note = C20DA-gGlu-gGlu-OEG-OEG
XVLSLDVPIGLLQILLSQARARAAREQAKTNNEILAEV

SEQ ID NO: 174 - protein, 38 aa, synthetic construct
  SITE 1: note = MeIle
  SITE 35: note = Nle
  LIPID 29: note = C20DA-gGlu-gGlu-OEG-OEG
XVLSLDVPIGLLQILLSQARARAAREQAKTNNEIXAEV

SEQ ID NO: 175 - protein, 38 aa, synthetic construct
  SITE 1: note = MeIle
  LIPID 29: note = C20DA-gGlu-gGlu-OEG-OEG
XVLSLDVPIGLLQILLSQARARAAREQAKTNDEILAEV

SEQ ID NO: 176 - protein, 38 aa, synthetic construct
  SITE 1: note = MeIle
  SITE 35: note = Nle
  LIPID 29: note = C20DA-gGlu-gGlu-OEG-OEG
XVLSLDVPIGLLQILLSQARARAAREQAKTNDEIXAEV

SEQ ID NO: 177 - protein, 38 aa, synthetic construct
  SITE 1: note = MeIle
  LIPID 29: note = C20DA-gGlu-gGlu-OEG-OEG
XVLSLDVPIGLLQILLSQARARAAREQAKTNQEILAEV

SEQ ID NO: 178 - protein, 38 aa, synthetic construct
  SITE 1: note = MeIle
  SITE 35: note = Nle
  LIPID 29: note = C20DA-gGlu-gGlu-OEG-OEG
XVLSLDVPIGLLQILLSQARARAAREQAKTNQEIXAEV

SEQ ID NO: 179 - protein, 38 aa, synthetic construct
  SITE 1: note = MeIle
  LIPID 29: note = C20DA-gGlu-gGlu-OEG-OEG
XVLSLDVPIGLLQILLSQARARAAREQAKTNGEILAEV

SEQ ID NO: 180 - protein, 38 aa, synthetic construct
  SITE 1: note = MeIle
  SITE 35: note = Nle
  LIPID 29: note = C20DA-gGlu-gGlu-OEG-OEG
XVLSLDVPIGLLQILLSQARARAAREQAKTNGEIXAEV

SEQ ID NO: 181 - protein, 38 aa, synthetic construct
  SITE 1: note = MeIle
  LIPID 29: note = C20DA-gGlu-gGlu-OEG-OEG
XVLSLDVPIGLLQILLSQARARAAREQAKTNHEILAEV

SEQ ID NO: 182 - protein, 38 aa, synthetic construct
  SITE 1: note = MeIle
  SITE 35: note = Nle
  LIPID 29: note = C20DA-gGlu-gGlu-OEG-OEG
XVLSLDVPIGLLQILLSQARARAAREQAKTNHEIXAEV

SEQ ID NO: 183 - protein, 38 aa, synthetic construct
  SITE 1: note = MeIle
  LIPID 29: note = C20DA-gGlu-gGlu-OEG-OEG
XVLSLDVPIGLLQILLSQARARAAREQAKTNLEILAEV

SEQ ID NO: 184 - protein, 38 aa, synthetic construct
  SITE 1: note = MeIle
  SITE 35: note = Nle
  LIPID 29: note = C20DA-gGlu-gGlu-OEG-OEG
XVLSLDVPIGLLQILLSQARARAAREQAKTNLEIXAEV

SEQ ID NO: 185 - protein, 38 aa, synthetic construct
  SITE 1: note = MeIle
  LIPID 29: note = C20DA-gGlu-gGlu-OEG-OEG
XVLSLDVPIGLLQILLSQARARAAREQAKTNKEILAEV

SEQ ID NO: 186 - protein, 38 aa, synthetic construct
  SITE 1: note = MeIle
  SITE 35: note = Nle
  LIPID 29: note = C20DA-gGlu-gGlu-OEG-OEG
XVLSLDVPIGLLQILLSQARARAAREQAKTNKEIXAEV

SEQ ID NO: 187 - protein, 38 aa, synthetic construct
  SITE 1: note = MeIle
  LIPID 29: note = C20DA-gGlu-gGlu-OEG-OEG
XVLSLDVPIGLLQILLSQARARAAREQAKTNFEILAEV

SEQ ID NO: 188 - protein, 38 aa, synthetic construct
  SITE 1: note = MeIle
  SITE 35: note = Nle
  LIPID 29: note = C20DA-gGlu-gGlu-OEG-OEG
XVLSLDVPIGLLQILLSQARARAAREQAKTNFEIXAEV

SEQ ID NO: 189 - protein, 38 aa, synthetic construct
  SITE 1: note = MeIle
  LIPID 29: note = C20DA-gGlu-gGlu-OEG-OEG
XVLSLDVPIGLLQILLSQARARAAREQAKTNSEILAEV

SEQ ID NO: 190 - protein, 38 aa, synthetic construct
  SITE 1: note = MeIle
  SITE 35: note = Nle
  LIPID 29: note = C20DA-gGlu-gGlu-OEG-OEG
XVLSLDVPIGLLQILLSQARARAAREQAKTNSEIXAEV

SEQ ID NO: 191 - protein, 38 aa, synthetic construct
  SITE 1: note = MeIle
  LIPID 29: note = C20DA-gGlu-gGlu-OEG-OEG
XVLSLDVPIGLLQILLSQARARAAREQAKTNTEILAEV

SEQ ID NO: 192 - protein, 38 aa, synthetic construct
  SITE 1: note = MeIle
  SITE 35: note = Nle
  LIPID 29: note = C20DA-gGlu-gGlu-OEG-OEG
XVLSLDVPIGLLQILLSQARARAAREQAKTNTEIXAEV

SEQ ID NO: 193 - protein, 38 aa, synthetic construct
  SITE 1: note = MeIle
  LIPID 29: note = C20DA-gGlu-gGlu-OEG-OEG
XVLSLDVPIGLLQILLSQARARAAREQAKTNWEILAEV

SEQ ID NO: 194 - protein, 38 aa, synthetic construct
  SITE 1: note = MeIle
  SITE 35: note = Nle
  LIPID 29: note = C20DA-gGlu-gGlu-OEG-OEG
XVLSLDVPIGLLQILLSQARARAAREQAKTNWEIXAEV

SEQ ID NO: 195 - protein, 38 aa, synthetic construct
  SITE 1: note = MeIle
  SITE 32: note = Aib
  LIPID 29: note = C20DA-gGlu-gGlu-OEG-OEG
XVLSLDVPIGLLQILLAQARARAAREQAKTNXEILAEV

SEQ ID NO: 196 - protein, 38 aa, synthetic construct
  SITE 1: note = MeIle
  SITE 32: note = Aib
  SITE 35: note = Nle
  LIPID 29: note = C20DA-gGlu-gGlu-OEG-OEG
XVLSLDVPIGLLQILLAQARARAAREQAKTNXEIXAEV

SEQ ID NO: 197 - protein, 38 aa, synthetic construct
  SITE 1: note = MeIle
  SITE 32: note = Aib
  LIPID 29: note = C20DA-gGlu-gGlu-OEG-OEG
XVLSLDVPIGLLQILLRQARARAAREQAKTNXEILAEV

SEQ ID NO: 198 - protein, 38 aa, synthetic construct
  SITE 1: note = MeIle
  SITE 32: note = Aib
  SITE 35: note = Nle
  LIPID 29: note = C20DA-gGlu-gGlu-OEG-OEG
XVLSLDVPIGLLQILLRQARARAAREQAKTNXEIXAEV

SEQ ID NO: 199 - protein, 38 aa, synthetic construct
  SITE 1: note = MeIle
  SITE 32: note = Aib
  LIPID 29: note = C20DA-gGlu-gGlu-OEG-OEG
XVLSLDVPIGLLQILLDQARARAAREQAKTNXEILAEV

SEQ ID NO: 200 - protein, 38 aa, synthetic construct
  SITE 1: note = MeIle
  SITE 32: note = Aib
  SITE 35: note = Nle
  LIPID 29: note = C20DA-gGlu-gGlu-OEG-OEG
XVLSLDVPIGLLQILLDQARARAAREQAKTNXEIXAEV

SEQ ID NO: 201 - protein, 38 aa, synthetic construct
  SITE 1: note = MeIle
  SITE 32: note = Aib
  LIPID 29: note = C20DA-gGlu-gGlu-OEG-OEG
XVLSLDVPIGLLQILLQQARARAAREQAKTNXEILAEV

SEQ ID NO: 202 - protein, 38 aa, synthetic construct
  SITE 1: note = MeIle
  SITE 32: note = Aib
  SITE 35: note = Nle
  LIPID 29: note = C20DA-gGlu-gGlu-OEG-OEG
XVLSLDVPIGLLQILLQQARARAAREQAKTNXEIXAEV

SEQ ID NO: 203 - protein, 38 aa, synthetic construct
  SITE 1: note = MeIle
  SITE 32: note = Aib
  LIPID 29: note = C20DA-gGlu-gGlu-OEG-OEG
XVLSLDVPIGLLQILLGQARARAAREQAKTNXEILAEV

SEQ ID NO: 204 - protein, 38 aa, synthetic construct
  SITE 1: note = MeIle
  SITE 32: note = Aib
  SITE 35: note = Nle
  LIPID 29: note = C20DA-gGlu-gGlu-OEG-OEG
XVLSLDVPIGLLQILLGQARARAAREQAKTNXEIXAEV

SEQ ID NO: 205 - protein, 38 aa, synthetic construct
  SITE 1: note = MeIle
  SITE 32: note = Aib
  SITE 35: note = Nle
  LIPID 29: note = C20DA-gGlu-gGlu-OEG-OEG
XVLSLDVPIGLLQILLEQARARAAREQAKTNXEIXAEV

SEQ ID NO: 206 - protein, 38 aa, synthetic construct
  SITE 1: note = MeIle
  SITE 32: note = Aib
  LIPID 29: note = C20DA-gGlu-gGlu-OEG-OEG
XVLSLDVPIGLLQILLHQARARAAREQAKTNXEILAEV

SEQ ID NO: 207 - protein, 38 aa, synthetic construct
  SITE 1: note = MeIle
  SITE 32: note = Aib
  SITE 35: note = Nle
  LIPID 29: note = C20DA-gGlu-gGlu-OEG-OEG
XVLSLDVPIGLLQILLHQARARAAREQAKTNXEIXAEV

SEQ ID NO: 208 - protein, 38 aa, synthetic construct
  SITE 1: note = MeIle
  SITE 32: note = Aib
  LIPID 29: note = C20DA-gGlu-gGlu-OEG-OEG
XVLSLDVPIGLLQILLIQARARAAREQAKTNXEILAEV

SEQ ID NO: 209 - protein, 38 aa, synthetic construct
  SITE 1: note = MeIle
  SITE 32: note = Aib
  SITE 35: note = Nle
  LIPID 29: note = C20DA-gGlu-gGlu-OEG-OEG
XVLSLDVPIGLLQILLIQARARAAREQAKTNXEIXAEV

SEQ ID NO: 210 - protein, 38 aa, synthetic construct
  SITE 1: note = MeIle
  SITE 32: note = Aib
  LIPID 29: note = C20DA-gGlu-gGlu-OEG-OEG
XVLSLDVPIGLLQILLFQARARAAREQAKTNXEILAEV

SEQ ID NO: 211 - protein, 38 aa, synthetic construct
  SITE 1: note = MeIle
  SITE 32: note = Aib
  SITE 35: note = Nle
  LIPID 29: note = C20DA-gGlu-gGlu-OEG-OEG
XVLSLDVPIGLLQILLFQARARAAREQAKTNXEIXAEV

SEQ ID NO: 212 - protein, 38 aa, synthetic construct
  SITE 1: note = MeIle
  SITE 32: note = Aib
  LIPID 29: note = C20DA-gGlu-gGlu-OEG-OEG
XVLSLDVPIGLLQILLPQARARAAREQAKTNXEILAEV

SEQ ID NO: 213 - protein, 38 aa, synthetic construct
  SITE 1: note = MeIle
  SITE 32: note = Aib
  SITE 35: note = Nle
  LIPID 29: note = C20DA-gGlu-gGlu-OEG-OEG
XVLSLDVPIGLLQILLPQARARAAREQAKTNXEIXAEV

SEQ ID NO: 214 - protein, 38 aa, synthetic construct
  SITE 1: note = MeIle
  SITE 32: note = Aib
  LIPID 29: note = C20DA-gGlu-gGlu-OEG-OEG
XVLSLDVPIGLLQILLSQARARAAREQAKTNXEILAEV

SEQ ID NO: 215 - protein, 38 aa, synthetic construct
  SITE 1: note = MeIle
  SITE 32: note = Aib
  SITE 35: note = Nle
  LIPID 29: note = C20DA-gGlu-gGlu-OEG-OEG
XVLSLDVPIGLLQILLSQARARAAREQAKTNXEIXAEV

SEQ ID NO: 216 - protein, 38 aa, synthetic construct
  SITE 1: note = MeIle
  SITE 32: note = Aib
  LIPID 29: note = C20DA-gGlu-gGlu-OEG-OEG
XVLSLDVPIGLLQILLTQARARAAREQAKTNXEILAEV

SEQ ID NO: 217 - protein, 38 aa, synthetic construct
  SITE 1: note = MeIle
  SITE 32: note = Aib
  SITE 35: note = Nle
  LIPID 29: note = C20DA-gGlu-gGlu-OEG-OEG
XVLSLDVPIGLLQILLTQARARAAREQAKTNXEIXAEV

SEQ ID NO: 218 - protein, 38 aa, synthetic construct
  SITE 1: note = MeIle
  SITE 32: note = Aib
  LIPID 29: note = C20DA-gGlu-gGlu-OEG-OEG
XVLSLDVPIGLLQILLWQARARAAREQAKTNXEILAEV

SEQ ID NO: 219 - protein, 38 aa, synthetic construct
  SITE 1: note = MeIle
  SITE 32: note = Aib
  SITE 35: note = Nle
  LIPID 29: note = C20DA-gGlu-gGlu-OEG-OEG
XVLSLDVPIGLLQILLWQARARAAREQAKTNXEIXAEV

SEQ ID NO: 220 - protein, 38 aa, synthetic construct
  SITE 1: note = MeIle
  SITE 32: note = Aib
  LIPID 29: note = C20DA-gGlu-gGlu-OEG-OEG
XVLSLDVPIGLLQILLYQARARAAREQAKTNXEILAEV

SEQ ID NO: 221 - protein, 38 aa, synthetic construct
  SITE 1: note = MeIle
  SITE 32: note = Aib
  SITE 35: note = Nle
  LIPID 29: note = C20DA-gGlu-gGlu-OEG-OEG
XVLSLDVPIGLLQILLYQARARAAREQAKTNXEIXAEV

SEQ ID NO: 222 - protein, 38 aa, synthetic construct
  SITE 1: note = MeIle
  SITE 32: note = Aib
  LIPID 29: note = C20DA-gGlu-gGlu-OEG-OEG
XVLSLDVPIGLLQILLEQARARAAREQAKTNXEILAEI

SEQ ID NO: 223 - protein, 38 aa, synthetic construct
  SITE 1: note = MeIle
  SITE 32: note = Aib
  SITE 35: note = Nle
  LIPID 29: note = C20DA-gGlu-gGlu-OEG-OEG
XVLSLDVPIGLLQILLEQARARAAREQAKTNXEIXAEI

SEQ ID NO: 224 - protein, 38 aa, synthetic construct
  SITE 1: note = MeIle
  SITE 32: note = Aib
  LIPID 29: note = C20DA-gGlu-gGlu-OEG-OEG
XVLSLDVPIGLLQILLEQARARAAREQAKTNXEILAEL

SEQ ID NO: 225 - protein, 38 aa, synthetic construct
  SITE 1: note = MeIle
  SITE 32: note = Aib
  SITE 35: note = Nle
  LIPID 29: note = C20DA-gGlu-gGlu-OEG-OEG
XVLSLDVPIGLLQILLEQARARAAREQAKTNXEIXAEL

SEQ ID NO: 226 - protein, 38 aa, synthetic construct
  SITE 1: note = MeIle
  SITE 32: note = Aib
  SITE 38: note = Aib
  LIPID 29: note = C20DA-gGlu-gGlu-OEG-OEG
XVLSLDVPIGLLQILLEQARARAAREQAKTNXEILAEX

SEQ ID NO: 227 - protein, 38 aa, synthetic construct
  SITE 1: note = MeIle
  SITE 32: note = Aib
  SITE 35: note = Nle
  SITE 38: note = Aib
  LIPID 29: note = C20DA-gGlu-gGlu-OEG-OEG
XVLSLDVPIGLLQILLEQARARAAREQAKTNXEIXAEX

SEQ ID NO: 228 - protein, 38 aa, synthetic construct
IVLSLDVPIGLLQILLEQARARAAREQATTNAEILAEV

SEQ ID NO: 229 - protein, 38 aa, synthetic construct
  SITE 1: note = MeIle
  SITE 32: note = Aib
  SITE 35: note = Nle
  LIPID 29: note = C20DA-gGlu-gGlu-OEG-OEG
XVLSLDVPIGLLQILLLQARARAAREQAKTNXEIXAEV

SEQ ID NO: 230 - protein, 38 aa, synthetic construct
  SITE 1: note = MeIle
  SITE 32: note = Aib
  SITE 35: note = Nle
  LIPID 29: note = C20DA-gGlu-gGlu-OEG-OEG
XVLSLDVPIGLLQILLKQARARAAREQAKTNXEIXAEV

SEQ ID NO: 231 - protein, 38 aa, synthetic construct
  SITE 1: note = MeIle
  SITE 32: note = Aib
  SITE 35: note = Nle
  LIPID 29: note = C20DA-gGlu-gGlu-OEG-OEG
XVLSLDVPIGLLQILLVQARARAAREQAKTNXEIXAEV

SEQ ID NO: 232 - protein, 38 aa, synthetic construct
  SITE 1: note = MeIle
  SITE 30: note = Aib
  SITE 35: note = Nle
  LIPID 29: note = C20DA-gGlu-gGlu-OEG-OEG
XVLSLDVPIGLLQILLRQARARAAREQAKXNAEIXAEV

SEQ ID NO: 233 - protein, 38 aa, synthetic construct
  SITE 1: note = MeIle
  SITE 30: note = Aib
  SITE 35: note = Nle
  LIPID 29: note = C20DA-gGlu-gGlu-OEG-OEG
XVLSLDVPIGLLQILLKQARARAAREQAKXNAEIXAEV

SEQ ID NO: 234 - protein, 38 aa, synthetic construct
  SITE 32: note = Aib
  SITE 35: note = Nle
  LIPID 29: note = C20DA-gGlu-gGlu-OEG-OEG
IVLSLDVPIGLLQILLSQARARAAREQAKTNXEIXAEV

SEQ ID NO: 235 - protein, 38 aa, synthetic construct
  SITE 1: note = MeIle
  SITE 30: note = Aib
  SITE 35: note = Nle
  LIPID 29: note = C20DA-gGlu-gGlu-OEG-OEG
XVLSLDVPIGLLQILLLQARARAAREQAKXNAEIXAEV

SEQ ID NO: 236 - protein, 38 aa, synthetic construct
  SITE 30: note = Aib
  SITE 35: note = Nle
  LIPID 29: note = C20DA-gGlu-gGlu-OEG-OEG
IVLSLDVPIGLLQILLEQARARAAREQAKXNAEIXAEI

SEQ ID NO: 237 - protein, 38 aa, synthetic construct
  SITE 30: note = Aib
  SITE 35: note = Nle
  LIPID 29: note = C20DA-gGlu-gGlu-OEG-OEG
IVLSLDVPIGLLQILLSQARARAAREQAKXNAEIXAEV

SEQ ID NO: 238 - protein, 38 aa, synthetic construct
  SITE 30: note = Aib
  SITE 35: note = Nle
  LIPID 29: note = C20DA-gGlu-gGlu-OEG-OEG
PVLSLDVPIGLLQILLSQARARAAREQAKXNAEIXAEV

SEQ ID NO: 239 - protein, 38 aa, synthetic construct
  SITE 35: note = Nle
  LIPID 29: note = C20DA-gGlu-gGlu-OEG-OEG
IVLSLDVPIGLLQILLSQARARAAREQAKENAEIXAEV

SEQ ID NO: 240 - protein, 38 aa, synthetic construct
  SITE 1: note = X = I, MeI or P
  SITE 3: note = X = L or T
  SITE 7: note = X = Cle or V
  SITE 8: note = X = P or Hyp
  SITE 9: note = X = I or L
  SITE 17: note = X = E, A, F, G, H, I, K, L, N, Q, R, S, T, D, P, W, Y or V
  SITE 18: note = X = Q, E or L
  SITE 19: note = X = A or E
  SITE 21: note = X = A, or E
  SITE 22: note = X = R, E or K
  SITE 23: note = X = A, E or L
  SITE 24: note = X = A, E, or K
  SITE 25: note = X = R, E, or K
  SITE 26: note = X = E or K
  SITE 27: note = X = Q or R
  SITE 29: note = X = T or K
  SITE 30: note = X = T, E, K, V, Y, W, S, P, F, L, I, H, G, Q, A or Aib
  SITE 32: note = X = A, E, W, T, S, F, K, L, H, G, Q, D, N, R, Aib, L, I, or V
  SITE 33: note = X = R or E
  SITE 35: note = X = L or Nle
  SITE 36: note = X = A or E
  SITE 37: note = X = R, E or K
  SITE 38: note = X = V, or I
XVXSLDXXXGLLQILLXXXRXXXXXXXAXXNXXIXXXX

SEQ ID NO: 241 - protein, 38 aa, synthetic construct
  SITE 1: note = X = I, MeI or P
  SITE 3: note = X = L or T
  SITE 7: note = X = Cle or V
  SITE 8: note = X = P or Hyp
  SITE 9: note = X = I or L
  SITE 17: note = X = E, A, F, G, H, I, K, L, N, Q, R, S, T, D, P, W, Y or V
  SITE 18: note = X = Q, or L
  SITE 19: note = X = A or E
  SITE 22: note = X = R, or K
  SITE 23: note = X = A, or L
  SITE 24: note = X = A, or K
  SITE 25: note = X = R, or K
  SITE 26: note = X = E or K
  SITE 27: note = X = Q or R
  SITE 29: note = X = T or K
  SITE 30: note = X = T, E, K, V, Y, W, S, P, F, L, I, H, G, Q, A or Aib
  SITE 32: note = X = A, E, W, T, S, F, K, L, H, G, Q, D, N, R, Aib, L, I, or V
  SITE 33: note = X = R or E
  SITE 35: note = L or Nle
  SITE 37: note = X = R, E or K
  SITE 38: note = X = V, or I
XVXSLDXXXGLLQILLXXXRAXXXXXXAXXNXXIXAXX

SEQ ID NO: 242 - protein, 38 aa, synthetic construct
  SITE 1: note = X = I, MeI or P
  SITE 3: note = X = L or T
  SITE 7: note = X = Cle or V
  SITE 8: note = X = P or Hyp
  SITE 9: note = X = I or L
  SITE 17: note = X = E, A, F, G, H, I, K, L, N, Q, R, S, T, D, P, W, Y or V
  SITE 18: note = X = Q or L
  SITE 19: note = X = A or E
  SITE 23: note = X = A, or L
  SITE 26: note = X = E or K
  SITE 27: note = X = Q or R
  SITE 29: note = X = T or K
  SITE 30: note = X = T, E, K, V, Y, W, S, P, F, L, I, H, G, Q, A or Aib
  SITE 32: note = X = A, E, W, T, S, F, K, L, H, G, Q, D, N, R, Aib, L, I, or V
  SITE 33: note = X = R or E
  SITE 35: note = X = L or Nle
  SITE 37: note = X = R, E or K
  SITE 38: note = X = V, or I
XVXSLDXXXGLLQILLXXXRARXARXXAXXNXXIXAXX

SEQ ID NO: 243 - protein, 38 aa, synthetic construct
  SITE 1: note = X = I, MeI or P
  SITE 3: note = X = L or T
  SITE 7: note = X = Cle or V
  SITE 8: note = X = P or Hyp
  SITE 9: note = X = I or L
  SITE 17: note = X = E, A, F, G, H, I, K, L, N, Q, R, S, T, D, P, W, Y or V
  SITE 18: note = X = Q or L
  SITE 23: note = X = A, or L
  SITE 26: note = X = E or K
  SITE 27: note = X = Q or R
  SITE 29: note = X = T or K
  SITE 30: note = X = T, E, K, V, Y, W, S, P, F, L, I, H, G, Q, A or Aib
  SITE 32: note = X = A, E, W, T, S, F, K, L, H, G, Q, D, N, R, Aib, L, I, or V
  SITE 35: note = X = L or Nle
  SITE 38: note = X = V, or I
XVXSLDXXXGLLQILLXXARARXARXXAXXNXEIXAEX

SEQ ID NO: 244 - protein, 38 aa, synthetic construct
  SITE 1: note = X = I, MeI or P
  SITE 3: note = X = L or T
  SITE 7: note = X = Cle or V
  SITE 8: note = X = P or Hyp
  SITE 9: note = X = I or L
  SITE 17: note = X = E, A, F, G, H, I, K, L, N, Q, R, S, T, D, P, W, Y or V
  SITE 18: note = X = Q or L
  SITE 23: note = X = A, or L
  SITE 27: note = X = Q or R
  SITE 29: note = X = T or K
  SITE 30: note = X = T, E, K, V, Y, W, S, P, F, L, I, H, G, Q, A or Aib
  SITE 32: note = X = A, E, W, T, S, F, K, L, H, G, Q, D, N, R, Aib, L, I, or V
  SITE 35: note = X = L or Nle
  SITE 38: note = X = V, or I
XVXSLDXXXGLLQILLXXARARXAREXAXXNXEIXAEX

SEQ ID NO: 245 - protein, 38 aa, synthetic construct; identical to SEQ ID NO: 240
  SITE 1: note = X = I, MeI or P
  SITE 3: note = X = L or T
  SITE 7: note = X = Cle or V
  SITE 8: note = X = P or Hyp
  SITE 9: note = X = I or L
  SITE 17: note = X = E, A, F, G, H, I, K, L, N, Q, R, S, T, D, P, W, Y or V
  SITE 18: note = X = Q, E or L
  SITE 19: note = X = A or E
  SITE 21: note = X = A, or E
  SITE 22: note = X = R, E or K
  SITE 23: note = X = A, E or L
  SITE 24: note = X = A, E, or K
  SITE 25: note = X = R, E, or K
  SITE 26: note = X = E or K
  SITE 27: note = X = Q or R
  SITE 29: note = X = T or K
  SITE 30: note = X = T, E, K, or Aib
  SITE 32: note = X = A, E, Aib, L, I, or V
  SITE 33: note = X = R or E
  SITE 35: note = X = L or Nle
  SITE 36: note = X = A or E
  SITE 37: note = X = R, E or K
  SITE 38: note = X = V, or I

SEQ ID NO: 246 - protein, 38 aa, synthetic construct; identical to SEQ ID NO: 243
  SITE 1: note = X = I, MeI or P
  SITE 3: note = X = L or T
  SITE 7: note = X = Cle or V
  SITE 8: note = X = P or Hyp
  SITE 9: note = X = I or L
  SITE 17: note = X = E, A, F, G, H, I, K, L, N, Q, R, S, T, D, P, W, Y or V
  SITE 18: note = X = Q or L
  SITE 23: note = X = A, or L
  SITE 26: note = X = E or K
  SITE 27: note = X = Q or R
  SITE 29: note = X = T or K
  SITE 30: note = X = T, E, K, or Aib
  SITE 32: note = X = A, Aib, L, I, or V
  SITE 35: note = X = L or Nle
  SITE 38: note = X = V, or I

SEQ ID NO: 247 - protein, 38 aa, synthetic construct; identical to SEQ ID NO: 244
  SITE 1: note = X = I, MeI or P
  SITE 3: note = X = L or T
  SITE 7: note = X = Cle or V
  SITE 8: note = X = P or Hyp
  SITE 9: note = X = I or L
  SITE 17: note = X = E, A, F, G, H, I, K, L, N, Q, R, S, T, D, P, W, Y or V
  SITE 18: note = X = Q or L
  SITE 23: note = X = A, or L
  SITE 27: note = X = Q or R
  SITE 29: note = X = T or K
  SITE 30: note = X = T, E, K, or Aib
  SITE 32: note = X = A, Aib, L, I, or V
  SITE 35: note = X = L or Nle
  SITE 38: note = X = V, or I

SEQ ID NO: 248 - protein, 38 aa, synthetic construct; identical to SEQ ID NO: 240
  SITE 1: note = X = I, MeI or P
  SITE 3: note = X = L or T
  SITE 7: note = X = Cle or V
  SITE 8: note = X = P or Hyp
  SITE 9: note = X = I or L
  SITE 17: note = X = E, A, F, G, H, I, K, L, N, Q, R, S, T, D, P, W, Y or V
  SITE 18: note = X = Q, E or L
  SITE 19: note = X = A or E
  SITE 21: note = X = A, or E
  SITE 22: note = X = R, E or K
  SITE 23: note = X = A, E or L
  SITE 24: note = X = A, E, or K
  SITE 25: note = X = R, E, or K
  SITE 26: note = X = E or K
  SITE 27: note = X = Q or R
  SITE 29: note = X = T or K
  SITE 30: note = X = T, E, K, V, Y, W, S, P, F, L, I, H, G, Q, A or Aib
  SITE 32: note = X = A, E, W, T, S, F, K, L, H, G, Q, D, N, R, Aib, L, I, or V
  SITE 33: note = X = R or E
  SITE 35: note = X = Nle
  SITE 36: note = X = A or E
  SITE 37: note = X = R, E or K
  SITE 38: note = X = V, or I

SEQ ID NO: 249 - protein, 38 aa, synthetic construct; identical to SEQ ID NO: 244
  SITE 1: note = X = I, MeI or P
  SITE 3: note = X = L or T
  SITE 7: note = X = Cle or V
  SITE 8: note = X = P or Hyp
  SITE 9: note = X = L or I
  SITE 17: note = X = E, A, F, G, H, I, K, L, N, Q, R, S, T, D, P, W, Y or V
  SITE 18: note = X = Q or L
  SITE 23: note = X = A, or L
  SITE 27: note = X = Q or R
  SITE 29: note = X = T or K
  SITE 30: note = X = T, E, K, V, Y, W, S, P, F, L, I, H, G, Q, A or Aib
  SITE 32: note = X = A, E, W, T, S, F, K, L, H, G, Q, D, N, R, Aib, L, I, or V
  SITE 35: note = X = Nle
  SITE 38: note = X = V, or I

SEQ ID NO: 250 - protein, 38 aa, synthetic construct; identical to SEQ ID NO: 244
  SITE 1: note = X = I, MeI or P
  SITE 3: note = X = L or T
  SITE 7: note = X = Cle or V
  SITE 8: note = X = P or Hyp
  SITE 9: note = X = L or I
  SITE 17: note = X = E, A, F, G, H, I, K, L, N, Q, R, S, T, D, P, W, Y or V
  SITE 18: note = X = Q or L
  SITE 23: note = X = A, or L
  SITE 27: note = X = Q or R
  SITE 29: note = X = T or K
  SITE 30: note = X = T, E, K, or Aib
  SITE 32: note = X = A, Aib, L, I, or V
  SITE 35: note = X = Nle
  SITE 38: note = X = V, or I

SEQ ID NO: 251 - protein, 38 aa, synthetic construct; identical to SEQ ID NO: 244
  SITE 1: note = X = I, MeI or P
  SITE 3: note = X = L or T
  SITE 7: note = X = Cle or V
  SITE 8: note = X = P or Hyp
  SITE 9: note = X = L or I
  SITE 17: note = X = E, A, F, G, H, I, K, L, N, Q, R, S, T, D, P, W, Y or V
  SITE 18: note = X = Q or L
  SITE 23: note = X = A, or L
  SITE 27: note = X = Q or R
  SITE 29: note = X = T or K
  SITE 30: note = X = T, E, K, V, Y, W, S, P, F, L, I, H, G, Q, A or Aib
  SITE 32: note = X = A, E, W, T, S, F, K, L, H, G, Q, D, N, R, Aib, L, I, or V
  SITE 35: note = X = Nle
  SITE 38: note = X = V, or I

SEQ ID NO: 252 - protein, 38 aa, synthetic construct; identical to SEQ ID NO: 244
  SITE 1: note = X = I, MeI or P
  SITE 3: note = X = L or T
  SITE 7: note = X = Cle or V
  SITE 8: note = X = P or Hyp
  SITE 9: note = X = L or I
  SITE 17: note = X = E, A, F, G, H, I, K, L, N, Q, R, S, T, D, P, W, Y or V
  SITE 18: note = X = Q or L
  SITE 23: note = X = A, or L
  SITE 27: note = X = Q or R
  SITE 29: note = X = T or K
  SITE 30: note = X = T, E, K, V, Y, W, S, P, F, L, I, H, G, Q, A or Aib
  SITE 32: note = X = A, E, W, T, S, F, K, L, H, G, Q, D, N, R, Aib, L, I, or V
  SITE 35: note = X = Nle
  SITE 38: note = X = V, or I

SEQ ID NO: 253 - protein, 38 aa, synthetic construct; identical to SEQ ID NO: 244
  SITE 1: note = X = I, MeI or P
  SITE 3: note = X = L or T
  SITE 7: note = X = Cle or V
  SITE 8: note = X = P or Hyp
  SITE 9: note = X = L or I
  SITE 17: note = X = E, A, F, G, H, I, K, L, N, Q, R, S, T, D, P, W, Y or V
  SITE 18: note = X = Q or L
  SITE 23: note = X = A, or L
  SITE 27: note = X = Q or R
  SITE 29: note = X = T or K
  SITE 30: note = X = T, E, K, or Aib
  SITE 32: note = X = A, Aib, L, I, or V
  SITE 35: note = X = Nle
  SITE 38: note = X = V, or I

SEQ ID NO: 254 - protein, 38 aa, synthetic construct
  SITE 1: note = X = I, MeI or P
  SITE 3: note = X = L or T
  SITE 7: note = X = Cle or V
  SITE 8: note = X = P or Hyp
  SITE 9: note = X = L or I
  SITE 17: note = X = E, A, F, G, H, I, K, L, N, Q, R, S, T, D, P, W, Y or V
  SITE 29: note = X = T or K
  SITE 30: note = X = T, E, K, V, Y, W, S, P, F, L, I, H, G, Q, A or Aib
  SITE 32: note = X = A, E, W, T, S, F, K, L, H, G, Q, D, N, R, Aib, L, I, or V
  SITE 35: note = X = Nle
  SITE 38: note = X = V, or I
XVXSLDXXXGLLQILLXQARARAAREQAXXNXEIXAEX

SEQ ID NO: 255 - protein, 38 aa, synthetic construct; identical to SEQ ID NO: 254
  SITE 1: note = X = I, MeI or P
  SITE 3: note = X = L or T
  SITE 7: note = X = Cle or V
  SITE 8: note = X = P or Hyp
  SITE 9: note = X = L or I
  SITE 17: note = X = E, A, F, G, H, I, K, L, N, Q, R, S, T, D, P, W, Y or V
  SITE 29: note = X = T or K
  SITE 30: note = X = T, E, K, or Aib
  SITE 32: note = X = A, Aib, L, I, or V
  SITE 35: note = X = Nle
  SITE 38: note = X = V, or I

SEQ ID NO: 256 - protein, 38 aa, synthetic construct
  SITE 1: note = X = I, MeI or P
  SITE 3: note = X = L or T
  SITE 7: note = X = Cle or V
  SITE 8: note = X = P or Hyp
  SITE 9: note = X = L or I
  SITE 17: note = X = A, F, G, H, I, K, L, N, Q, R, S, T, or V
  SITE 18: note = X = Q or L
  SITE 23: note = X = A, or L
  SITE 27: note = X = Q or R
  SITE 29: note = X = T or K
  SITE 30: note = X = T, E, K, V, Y, W, S, P, F, L, I, H, G, Q, A or Aib
  SITE 32: note = X = A, E, W, T, S, F, K, L, H, G, Q, D, N, R, Aib, L, I, or V
  SITE 35: note = X = Nle
XVXSLDXXXGLLQILLXXARARXAREXAXXNXEIXAEV

SEQ ID NO: 257 - protein, 38 aa, synthetic construct
  SITE 1: note = X = I, MeI or P
  SITE 3: note = X = L or T
  SITE 7: note = X = Cle or V
  SITE 8: note = X = P or Hyp
  SITE 9: note = X = L or I
  SITE 17: note = X = A, F, G, H, I, K, L, N, Q, R, S, T, or V
  SITE 29: note = X = T or K
  SITE 30: note = X = T, E, K, or Aib
  SITE 32: note = X = A, Aib, L, I, or V
  SITE 35: note = X = Nle
XVXSLDXXXGLLQILLXQARARAAREQAXXNXEIXAEV

SEQ ID NO: 258 - protein, 38 aa, synthetic construct
  SITE 1: note = X = MeI or P
  SITE 17: note = X = N, F, G, K, Q, S, or T
  SITE 29: note = X = T or K
  SITE 30: note = X = T, E, K, or Aib
  SITE 32: note = X = A, Aib, L, I, or V
  SITE 35: note = X = Nle
XVLSLDVPIGLLQILLXQARARAAREQAXXNXEIXAEV

SEQ ID NO: 259 - protein, 38 aa, synthetic construct; identical to SEQ ID NO: 258
  SITE 1: note = X = MeI or P
  SITE 17: note = X = N, F, G, K, Q, S, or T
  SITE 30: note = X = T, or Aib
  SITE 32: note = X = A, or Aib
  SITE 35: note = X = Nle
  SITE 29: note = X = K*, wherein * denotes a covalent attachment of a lipid, optionally through a linker/spacer.

SEQ ID NO: 260 - protein, 38 aa, synthetic construct; identical to SEQ ID NO: 228
  LIPID 1: note = Lipid = C20DA-gGlu-gGlu-OEG-OEG

SEQ ID NO: 261 - protein, 38 aa, synthetic construct
  LIPID 12: note = Lipid = C20DA-gGlu-gGlu-OEG-OEG
IVLSLDVPIGLKQILLEQARARAAREQATTNAEILAEV

SEQ ID NO: 262 - protein, 38 aa, synthetic construct
  SITE 1: note = X = I, MeI or P
  SITE 17: note = X = E, A, F, G, H, I, K, L, N, Q, R, S, T, or V
  SITE 18: note = X = Q or L
  SITE 29: note = X = T or K
  SITE 30: note = X = T, E, K, V, Y, W, S, P, F, L, I, H, G, Q, A or Aib
  SITE 32: note = X = A, E, W, T, S, F, K, L, H, G, Q, D, N, R, Aib, L, I, or V
  SITE 35: note = X = L or Nle
  SITE 38: note = X = V or I
XVLSLDVPIGLLQILLXXARARAAREQAXXNXEIXAEX